European Patent Specification EP 3 749 338 B1, published July 17, 2024. Title: HUMANIZED BCMA ANTIBODY AND BCMA-CAR-T CELLS. Applicant: Caribou Biosciences, Inc. The sequence listing filed with the application follows.

SEQUENCE LISTING (17 sequences)

SEQ ID NO: 1 - protein, 184 aa, Homo sapiens
MLQMAGQCSQNEYFDSLLHACIPCQLRCSSNTPPLTCQRYCNASVTNSVKGTNAILWTCLGLSLIISLAVFVLMFLLRKINSEPLKDEFKNTGSGLLGMANIDLEKSRTGDEIILPRGLEYTVEECTCEDCIKSKPKVDSDHCFPLPAMEEGATILVTTKTNDYCKSLPAALSATEIEKSISAR

SEQ ID NO: 2 - DNA, 720 bp, Homo sapiens
caggtgcagctggtgcagagcggcgcggaagtgaaaaaaccgggcagcagcgtgaaagtgagctgcaaagcgagcggctatacctttaccagctatgtgatgcattgggtgcgccaggcgccgggccagggcctggaatggatgggctatattattccgtataacgatgcgaccaaatataacgaaaaatttaaaggccgcgtgaccattaccgcggataaaagcaccagcaccgcgtatatggaactgagcagcctgcgcagcgaagataccgcggtgtattattgcgcgcgctataactatgatggctattttgatgtgtggggccagggcaccctggtgaccgtgagcagcggcggcggcggcagcggcggcggcggcagcggcggcggcggcagcgaaattgtgctgacccagagcccggcgaccctgagcctgagcccgggcgaacgcgcgaccctgagctgccgcgcgagccagagcattagcgattatctgcattggtatcagcagaaaccgggccaggcgccgcgcctgctgatttattatgcgagccagagcattaccggcattccggcgcgctttagcggcagcggcagcggcaccgattttaccctgaccattagcagcctggaaccggaagattttgcggtgtattattgccagaacggccatagctttccgccgacctttggcggcggcaccaaagtggaaattaaa

SEQ ID NO: 3 - protein, 118 aa, Homo sapiens
QVQLVQSGAEVKKPGSSVKVSCKASGYTFTSYVMHWVRQAPGQGLEWMGYIIPYNDATKYNEKFKGRVTITADKSTSTAYMELSSLRSEDTAVYYCARYNYDGYFDVWGQGTLVTVSS

SEQ ID NO: 4 - protein, 15 aa, Artificial Sequence
  synthetic
GGGGSGGGGSGGGGS

SEQ ID NO: 5 - protein, 107 aa, Homo sapiens
EIVLTQSPATLSLSPGERATLSCRASQSISDYLHWYQQKPGQAPRLLIYYASQSITGIPARFSGSGSGTDFTLTISSLEPEDFAVYYCQNGHSFPPTFGGGTKVEIK

SEQ ID NO: 6 - protein, 240 aa, Homo sapiens
QVQLVQSGAEVKKPGSSVKVSCKASGYTFTSYVMHWVRQAPGQGLEWMGYIIPYNDATKYNEKFKGRVTITADKSTSTAYMELSSLRSEDTAVYYCARYNYDGYFDVWGQGTLVTVSSGGGGSGGGGSGGGGSEIVLTQSPATLSLSPGERATLSCRASQSISDYLHWYQQKPGQAPRLLIYYASQSITGIPARFSGSGSGTDFTLTISSLEPEDFAVYYCQNGHSFPPTFGGGTKVEIK

SEQ ID NO: 7 - DNA, 63 bp, Homo sapiens
atggccttaccagtgaccgccttgctcctgccgctggccttgctgctccacgccgccaggccg

SEQ ID NO: 8 - protein, 21 aa, Homo sapiens
MALPVTALLLPLALLLHAARP

SEQ ID NO: 9 - DNA, 141 bp, Homo sapiens
aagcccaccacgacgccagcgccgcgaccaccaacaccggcgcccaccatcgcgtcgcagcccctgtccctgcgcccagaggcgagccggccagcggcggggggcgcagtgcacacgagggggctggacttcgccagtgat

SEQ ID NO: 10 - protein, 47 aa, Homo sapiens
KPTTTPAPRPPTPAPTIASQPLSLRPEASRPAAGGAVHTRGLDFASD

SEQ ID NO: 11 - DNA, 81 bp, Homo sapiens
ttttgggtgctggtggtggttggtggagtcctggcttgctatagcttgctagtaacagtggcctttattattttctgggtg

SEQ ID NO: 12 - protein, 27 aa, Homo sapiens
FWVLVVVGGVLACYSLLVTVAFIIFWV

SEQ ID NO: 13 - DNA, 123 bp, Homo sapiens
aggagtaagaggagcaggctcctgcacagtgactacatgaacatgactccccgccgccccgggcccacccgcaagcattaccagccctatgccccaccacgcgacttcgcagcctatcgctcc

SEQ ID NO: 14 - protein, 41 aa, Homo sapiens
RSKRSRLLHSDYMNMTPRRPGPTRKHYQPYAPPRDFAAYRS

SEQ ID NO: 15 - DNA, 345 bp, Homo sapiens
agagtgaagttcagcaggagcgcagacgcccccgcgtaccagcagggccagaaccagctctataacgagctcaatctaggacgaagagaggagtacgatgttttggacaagagacgtggccgggaccctgagatggggggaaagccgcagagaaggaagaaccctcaggaaggcctgtacaatgaactgcagaaagataagatggcggaggcctacagtgagattgggatgaaaggcgagcgccggaggggcaaggggcacgatggcctttaccagggtctcagtacagccaccaaggacacctacgacgcccttcacatgcaggccctgccccctcgctaatag

SEQ ID NO: 16 - protein, 113 aa, Homo sapiens
RVKFSRSADAPAYQQGQNQLYNELNLGRREEYDVLDKRRGRDPEMGGKPQRRKNPQEGLYNELQKDKMAEAYSEIGMKGERRRGKGHDGLYQGLSTATKDTYDALHMQALPPR

SEQ ID NO: 17 - protein, 495 aa, Homo sapiens
MALPVTALLLPLALLLHAARPASQVQLVQSGAEVKKPGSSVKVSCKASGYTFTSYVMHWVRQAPGQGLEWMGYIIPYNDATKYNEKFKGRVTITADKSTSTAYMELSSLRSEDTAVYYCARYNYDGYFDVWGQGTLVTVSSGGGGSGGGGSGGGGSEIVLTQSPATLSLSPGERATLSCRASQSISDYLHWYQQKPGQAPRLLIYYASQSITGIPARFSGSGSGTDFTLTISSLEPEDFAVYYCQNGHSFPPTFGGGTKVEIKLEKPTTTPAPRPPTPAPTIASQPLSLRPEASRPAAGGAVHTRGLDFASDKPFWVLVVVGGVLACYSLLVTVAFIIFWVRSKRSRLLHSDYMNMTPRRPGPTRKHYQPYAPPRDFAAYRSRVKFSRSADAPAYQQGQNQLYNELNLGRREEYDVLDKRRGRDPEMGGKPQRRKNPQEGLYNELQKDKMAEAYSEIGMKGERRRGKGHDGLYQGLSTATKDTYDALHMQALPPR